European Patent Application EP 4 206 317 A1, published July 5, 2023. Title: Antitumor bacterial strains, and compositions and methods using the same. Applicant: Medytox Inc. The sequence listing filed with the application follows.

SEQUENCE LISTING (13 sequences)

SEQ ID NO: 1 - DNA, 20 bp, Artificial Sequence
  Primer
agagtttgatcmtggctcag

SEQ ID NO: 2 - DNA, 22 bp, Artificial Sequence
  Primer
tacggytaccttgttacgactt

SEQ ID NO: 3 - DNA, 1362 bp, Enterococcus faecium
aaaaagaggagtggcgaacgggtgagtaacacgtgggtaacctcgcccatcagaaggggataacacttggaaacaggtgctaataccgtataacaatcaaaaccgcatggttttgatttgaaaggcgctttcgggtgtcgctgatggatggacccgcggtgcattagctagttggtgaggtaacggctcaccaaggccacgatgcatagccgacctgagagggtgatcggccacattgggactgagacacggcccaaactcctacgggaggcagcagtagggaatcttcggcaatggacgaaagtctgaccgagcaacgccgcgtgagtgaagaaggttttcggatcgtaaaactctgttgttagagaagaacaaggatgagagtaactgttcatcccttgacggtatctaaccagaaagccacggctaactacgtgccagcagccgcggtaatacgtaggtggcaagcgttgtccggatttattgggcgtaaagcgagcgcaggcggtttcttaagtctgatgtgaaagcccccggctcaaccggggagggtcattggaaactgggagacttgagtgcagaagaggagagtggaattccatgtgtagcggtgaaatgcgtagatatatggaggaacaccagtggcgaaggcggctctctggtctgtaactgacgctgaggctcgaaagcgtggggagcaaacaggattagataccctggtagtccacgccgtaaacgatgagtgctaagtgttggagggtttccgcccttcagtgctgcagctaacgcattaagcactccgcctggggagtacgaccgcaaggttgaaactcaaaggaattgacgggggcccgcacaagcggtggagcatgtggtttaattcgaagcaacgcgaagaaccttaccaggtcttgacatcctttgaccactctagagatagagcttccccttcgggggcaaagtgacaggtggtgcatggttgtcgtcagctcgtgtcgtgagatgttgggttaagtcccgcaacgagcgcaacccttattgttagttgccatcattcagttgggcactctagcaagactgccggtgacaaaccggaggaaggtggggatgacgtcaaatcatcatgccccttatgacctgggctacacacgtgctacaatgggaagtacaacgagttgcgaagtcgcgaggctaagctaatctcttaaagcttctctcagttcggattgcaggctgcaactcgcctgcatgaagccggaatcgctagtaatcgcggatcagcacgccgcggtgaatacgttcccgggccttgtacacaccgcccgtcacaccacgagagtttgtaacacccgaagtcggtga

SEQ ID NO: 4 - DNA, 1391 bp, Enterococcus faecium
cgcttctttttccaccggagcttgctccaccggaaaaagaagagtggcgaacgggtgagtaacacgtgggtaacctgcccatcagaaggggataacacttggaaacaggtgctaataccgtataacaatcaaaaccgcatggttttgatttgaaaggcgctttcgggtgtcgctgatggatggacccgcggtgcattagctagttggtgaggtaacggctcaccaaggccacgatgcatagccgacctgagagggtgatcggccacattgggactgagacacggcccaaactcctacgggaggcagcagtagggaatcttcggcaatggacgaaagtctgaccgagcaacgccgcgtgagtgaagaaggttttcggatcgtaaaactctgttgttagagaagaacaaggatgagagtaactgttcatcccttgacggtatctaaccagaaagccacggctaactacgtgccagcagccgcggtaatacgtaggtggcaagcgttgtccggatttattgggcgtaaagcgagcgcaggcggtttcttaagtctgatgtgaaagcccccggctcaaccggggagggtcattggaaactgggagacttgagtgcagaagaggagagtggaattccatgtgtagcggtgaaatgcgtagatatatggaggaacaccagtggcgaaggcggctctctggtctgtaactgacgctgaggctcgaaagcgtggggagcaaacaggattagataccctggtagtccacgccgtaaacgatgagtgctaagtgttggagggtttccgcccttcagtgctgcagctaacgcattaagcactccgcctggggagtacgaccgcaaggttgaaactcaaaggaattgacgggggcccgcacaagcggtggagcatgtggtttaattcgaagcaacgcgaagaaccttaccaggtcttgacatcctttgaccactctagagatagagcttccccttcgggggcaaagtgacaggtggtgcatggttgtcgtcagctcgtgtcgtgagatgttgggttaagtcccgcaacgagcgcaacccttattgttagttgccatcattcagttgggcccccccccaagactgccggtgacaaaccggaggaaggtggggatgacgtcaaatcatcatgccccttatgacctgggctacacacgtgctacaatgggaagtacaacgagttgcgaagtcgcgaggctaagctaatctcttaaagcttctctcagttcggattgcaggctgcaactcgcctgcatgaagccggaatcgctagtaatcgcggatcagcacgccgcggtgaatacgttcccgggccttgtacacaccgcccgtcacaccacgagagtttgtaacacccgaagtcgg

SEQ ID NO: 5 - DNA, 1352 bp, Enterococcus faecium
aagaggagtggcgaacgggtgagtaacacgtgggtaacctgcccatcagaaggggataacacttggaaacaggtgctaataccgtataacaatcgaaaccgcatggttttgatttgaaaggcgctttcgggtgtcgctgatggatggacccgcggtgcattagctagttggtgaggtaacggctcaccaaggccacgatgcatagccgacctgagagggtgatcggccacattgggactgagacacggcccaaactcctacgggaggcagcagtagggaatcttcggcaatggacgaaagtctgaccgagcaacgccgcgtgagtgaagaaggttttcggatcgtaaaactctgttgttagagaagaacaaggatgagagtaactgttcatcccttgacggtatctaaccagaaagccacggctaactacgtgccagcagccgcggtaatacgtaggtggcaagcgttgtccggatttattgggcgtaaagcgagcgcaggcggtttcttaagtctgatgtgaaagcccccggctcaaccggggagggtcattggaaactgggagacttgagtgcagaagaggagagtggaattccatgtgtagcggtgaaatgcgtagatatatggaggaacaccagtggcgaaggcggctctctggtctgtaactgacgctgaggctcgaaagcgtggggagcaaacaggattagataccctggtagtccacgccgtaaacgatgagtgctaagtgttggagggtttccgcccttcagtgctgcagctaacgcattaagcactccgcctggggagtacgaccgcaaggttgaaactcaaaggaattgacgggggcccgcacaagcggtggagcatgtggtttaattcgaagcaacgcgaagaaccttaccaggtcttgacatcctttgaccactctagagatagagcttccccttcgggggcaaagtgacaggtggtgcatggttgtcgtcagctcgtgtcgtgagatgttgggttaagtcccgcaacgagcgcaacccttattgttagttgccatcattcagttgggcactctagcaagactgccggtgacaaaccggaggaaggtggggatgacgtcaaatcatcatgccccttatgacctgggctacacacgtgctacaatgggaagtacaacgagttgcgaagtcgcgaggctaagctaatctcttaaagcttctctcagttcggattgcaggctgcaactcgcctgcatgaagccggaatcgctagtaatcgcggatcagcacgccgcggtgaatacgttcccgggccttgtacacaccgcccgtcacaccacgagagtttgtaacacccgaagt

SEQ ID NO: 6 - DNA, 1388 bp, Enterococcus faecium
gcttctttttccaccggagcttgctccaccggaaaaagaggagtggcgaacgggtgagtaacacgtgggtaacctgcccatcagaaggggataacacttggaaacaggtgctaataccgtataacaatcgaaaccgcatggttttgatttgaaaggcgctttcgggtgtcgctgatggatggacccgcggtgcattagctagttggtgaggtaacggctcaccaaggccacgatgcatagccgacctgagagggtgatcggccacattgggactgagacacggcccaaactcctacgggaggcagcagtagggaatcttcggcaatggacgaaagtctgaccgagcaacgccgcgtgagtgaagaaggttttcggatcgtaaaactctgttgttagagaagaacaaggatgagagtaactgttcatcccttgacggtatctaaccagaaagccacggctaactacgtgccagcagccgcggtaatacgtaggtggcaagcgttgtccggatttattgggcgtaaagcgagcgcaggcggtttcttaagtctgatgtgaaagcccccggctcaaccggggagggtcattggaaactgggagacttgagtgcagaagaggagagtggaattccatgtgtagcggtgaaatgcgtagatatatggaggaacaccagtggcgaaggcggctctctggtctgtaactgacgctgaggctcgaaagcgtggggagcaaacaggattagataccctggtagtccacgccgtaaacgatgagtgctaagtgttggagggtttccgcccttcagtgctgcagctaacgcattaagcactccgcctggggagtacgaccgcaaggttgaaactcaaaggaattgacgggggcccgcacaagcggtggagcatgtggtttaattcgaagcaacgcgaagaaccttaccaggtcttgacatcctttgaccactctagagatagagcttccccttcgggggcaaagtgacaggtggtgcatggttgtcgtcagctcgtgtcgtgagatgttgggttaagtcccgcaacgagcgcaacccttattgttagttgccatcattcagttgggcactctagcaagactgccggtgacaaaccggaggaaggtggggatgacgtcaaatcatcatgccccttatgacctgggctacacacgtgctacaatgggaagtacaacgagttgcgaagtcgcgaggctaagctaatctcttaaagcttctctcagttcggattgcaggctgcaactcgcctgcatgaagccggaatcgctagtaatcgcggatcagcacgccgcggtgaatacgttcccgggccttgtacacaccgcccgtcacaccacgagagtttgtaacacccgaagtc

SEQ ID NO: 7 - DNA, 1389 bp, Enterococcus faecium
ggagcttgctccaccggaaaaagaggagtggcgaacgggtgagtaacacgtgggtaacctgcccatcagaaggggataacacttggaaacaggtgctaataccgtataacaatcaaaaccgcatggttttgatttgaaaggcgctttcgggtgtcgctgatggatggacccgcggtgcattagctagttggtgaggtaacggctcaccaaggccacgatgcatagccgacctgagagggtgatcggccacattgggactgagacacggcccaaactcctacgggaggcagcagtagggaatcttcggcaatggacgaaagtctgaccgagcaacgccgcgtgagtgaagaaggttttcggatcgtaaaactctgttgttagagaagaacaaggatgagagtaactgttcatcccttgacggtatctaaccagaaagccacggctaactacgtgccagcagccgcggtaatacgtaggtggcaagcgttgtccggatttattgggcgtaaagcgagcgcaggcggtttcttaagtctgatgtgaaagcccccggctcaaccggggagggtcattggaaactgggagacttgagtgcagaagaggagagtggaattccatgtgtagcggtgaaatgcgtagatatatggaggaacaccagtggcgaaggcggctctctggtctgtaactgacgctgaggctcgaaagcgtggggagcaaacaggattagataccctggtagtccacgccgtaaacgatgagtgctaagtgttggagggtttccgcccttcagtgctgcagctaacgcattaagcactccgcctggggagtacgaccgcaaggttgaaactcaaaggaattgacgggggcccgcacaagcggtggagcatgtggtttaattcgaagcaacgcgaagaaccttaccaggtcttgacatcctttgaccactctagagatagagcttccccttcgggggcaaagtgacaggtggtgcatggttgtcgtcagctcgtgtcgtgagatgttgggttaagtcccgcaacgagcgcaacccttattgttagttgccatcattcagttgggcactctagcaagactgccggtgacaaaccggaggaaggtggggatgacgtcaaatcatcatgccccttatgacctgggctacacacgtgctacaatgggaagtacaacgagtcgcgaagtcgcgaggctaagctaatctcttaaagcttctctcagttcggattgcaggctgcaactcgcctgcatgaagccggaatcgctagtaatcgcggatcagcacgccgcggtgaatacgttcccgggccttgtacacaccgcccgtcacaccacgagagtttgtaacacccgaagtcggtgaggtaacctttt

SEQ ID NO: 8 - DNA, 1358 bp, Enterococcus faecium
gaaaaagaggagtggcgaacgggtgagtaacacgtgggtaacctgcccatcagaaggggataacacttggaaacaggtgctaataccgtataacaatcgaaaccgcatggttttgatttgaaaggcgctttcgggtgtcgctgatggatggacccgcggtgcattagctagttggtgaggtaacggctcaccaaggccacgatgcatagccgacctgagagggtgatcggccacattgggactgagacacggcccaaactcctacgggaggcagcagtagggaatcttcggcaatggacgaaagtctgaccgagcaacgccgcgtgagtgaagaaggttttcggatcgtaaaactctgttgttagagaagaacaaggatgagagtaactgttcatcccttgacggtatctaaccagaaagccacggctaactacgtgccagcagccgcggtaatacgtaggtggcaagcgttgtccggatttattgggcgtaaagcgagcgcaggcggtttcttaagtctgatgtgaaagcccccggctcaaccggggagggtcattggaaactgggagacttgagtgcagaagaggagagtggaattccatgtgtagcggtgaaatgcgtagatatatggaggaacaccagtggcgaaggcggctctctggtctgtaactgacgctgaggctcgaaagcgtggggagcaaacaggattagataccctggtagtccacgccgtaaacgatgagtgctaagtgttggagggtttccgcccttcagtgctgcagctaacgcattaagcactccgcctggggagtacgaccgcaaggttgaaactcaaaggaattgacgggggcccgcacaagcggtggagcatgtggtttaattcgaagcaacgcgaagaaccttaccaggtcttgacatcctttgaccactctagagatagagcttccccttcgggggcaaagtgacaggtggtgcatggttgtcgtcagctcgtgtcgtgagatgttgggttaagtcccgcaacgagcgcaacccttattgttagttgccatcattcagttgggcactctagcaagactgccggtgacaaaccggaggaaggtggggatgacgtcaaatcatcatgccccttatgacctgggctacacacgtgctacaatgggaagtacaacgagttgcgaagtcgcgaggctaagctaatctcttaaagcttctctcagttcggattgcaggctgcaactcgcctgcatgaagccggaatcgctagtaatcgcggatcagcacgccgcggtgaatacgttcccgggccttgtacacaccgcccgtcacaccacgagagtttgtaacacccgaagtcg

SEQ ID NO: 9 - DNA, 1372 bp, Enterococcus faecium
ttctttttccaccggagcttgctccaccggaaaaagaagagtggcgaacgggtgagtaacacgtgggtaacctgcccatcagaaggggataacacttggaaacaggtgctaataccgtataacaatcaaaaccgcatggttttgatttgaaaggcgctttcgggtgtcgctgatggatggacccgcggtgcattagctagttggtgaggtaacggctcaccaaggccacgatgcatagccgacctgagagggtgatcggccacattgggactgagacacggcccaaactcctacgggaggcagcagtagggaatcttcggcaatggacgaaagtctgaccgagcaacgccgcgtgagtgaagaaggttttcggatcgtaaaactctgttgttagagaagaacaaggatgagagtaactgttcatcccttgacggtatctaaccagaaagccacggctaactacgtgccagcagccgcggtaatacgtaggtggcaagcgttgtccggatttattgggcgtaaagcgagcgcaggcggtttcttaagtctgatgtgaaagcccccggctcaaccggggagggtcattggaaactgggagacttgagtgcagaagaggagagtggaattccatgtgtagcggtgaaatgcgtagatatatggaggaacaccagtggcgaaggcggctctctggtctgtaactgacgctgaggctcgaaagcgtggggagcaaacaggattagataccctggtagtccacgccgtaaacgatgagtgctaagtgttggagggtttccgcccttcagtgctgcagctaacgcattaagcactccgcctggggagtacgaccgcaaggttgaaactcaaaggaattgacgggggcccgcacaagcggtggagcatgtggtttaattcgaagcaacgcgaagaaccttaccaggtcttgacatcctttgaccactctagagatagagcttccccttcgggggcaaagtgacaggtggtgcatggttgtcgtcagctcgtgtcgtgagatgttgggttaagtcccgcaacgagcgcaacccttattgttagttgccatcattcagttgggcactctagcaagactgccggtgacaaaccggaggaaggtggggatgacgtcaaatcatcatgccccttatgacctgggctacacacgtgctacaatgggaagtacaacgagttgcgaagtcgcgaggctaagctaatctcttaaagcttctctcagttcggattgcaggctgcaactcgcctgcatgaagccggaatcgctagtaatcgcggatcagcacgccgcggtgaatacgttcccgggccttgtacacaccgcccgtcacaccacgagagtttg

SEQ ID NO: 10 - DNA, 1381 bp, Enterococcus faecium
ggagcttgcttccaccggaaaaagaggagtggcgaacgggtgagtaacacgtgggtaacctgcccatcagaaggggataacacttggaaacaggtgctaataccgtataacaatcgaaaccgcatggttttgatttgaaaggcgctttcgggtgtcgctgatggatggacccgcggtgcattagctagttggtgaggtaacggctcaccaaggccacgatgcatagccgacctgagagggtgatcggccacattgggactgagacacggcccaaactcctacgggaggcagcagtagggaatcttcggcaatggacgaaagtctgaccgagcaacgccgcgtgagtgaagaaggttttcggatcgtaaaactctgttgttagagaagaacaaggatgagagtaactgttcatcccttgacggtatctaaccagaaagccacggctaactacgtgccagcagccgcggtaatacgtaggtggcaagcgttgtccggatttattgggcgtaaagcgagcgcaggcggtttcttaagtctgatgtgaaagcccccggctcaaccggggagggtcattggaaactgggagacttgagtgcagaagaggagagtggaattccatgtgtagcggtgaaatgcgtagatatatggaggaacaccagtggcgaaggcggctctctggtctgtaactgacgctgaggctcgaaagcgtggggagcaaacaggattagataccctggtagtccacgccgtaaacgatgagtgctaagtgttggagggtttccgcccttcagtgctgcagctaacgcattaagcactccgcctggggagtacgaccgcaaggttgaaactcaaaggaattgacgggggcccgcacaagcggtggagcatgtggtttaattcgaagcaacgcgaagaaccttaccaggtcttgacatcctttgaccactctagagatagagcttccccttcgggggcaaagtgacaggtggtgcatggttgtcgtcagctcgtgtcgtgagatgttgggttaagtcccgcaacgagcgcaacccttattgttagttgccatcattcagttgggcactctagcaagactgccggtgacaaaccggaggaaggtggggatgacgtcaaatcatcatgccccttatgacctgggctacacacgtgctacaatgggaagtacaacgagttgcgaagtcgcgaggctaagctaatctcttaaagcttctctcagttcggattgcaggctgcaactcgcctgcatgaagccggaatcgctagtaatcgcggatcagcacgccgcggtgaatacgttcccgggccttgtacacaccgcccgtcacaccacgagagtttgtaacacccgaagtcggtgagg

SEQ ID NO: 11 - DNA, 20 bp, Artificial Sequence
  primer
agagtttgatcmtggctcag

SEQ ID NO: 12 - DNA, 22 bp, Artificial Sequence
  primer
tacggytaccttgttacgactt

SEQ ID NO: 13 - DNA, 1339 bp, Enterococcus faecalis
agtgcttgcactcaattggaaagaggagtggcggacgggtgagtaacacgtgggtaacctacccatcagagggggataacacttggaaacaggtgctaataccgcataacagtttatgccgcatggcataagagtgaaaggcgctttcgggtgtcgctgatggatggacccgcggtgcattagctagttggtgaggtaacggctcaccaaggccacgatgcatagccgacctgagagggtgatcggccacactgggactgagacacggcccagactcctacgggaggcagcagtagggaatcttcggcaatggacgaaagtctgaccgagcaacgccgcgtgagtgaagaaggttttcggatcgtaaaactctgttgttagagaagaacaaggacgttagtaactgaacgtcccctgacggtatctaaccagaaagccacggctaactacgtgccagcagccgcggtaatacgtaggtggcaagcgttgtccggatttattgggcgtaaagcgagcgcaggcggtttcttaagtctgatgtgaaagcccccggctcaaccggggagggtcattggaaactgggagacttgagtgcagaagaggagagtggaattccatgtgtagcggtgaaatgcgtagatatatggaggaacaccagtggcgaaggcggctctctggtctgtaactgacgctgaggctcgaaagcgtggggagcaaacaggattagataccctggtagtccacgccgtaaacgatgagtgctaagtgttggagggtttccgcccttcagtgctgcagcaaacgcattaagcactccgcctggggagtacgaccgcaaggttgaaactcaaaggaattgacgggggcccgcacaagcggtggagcatgtggtttaattcgaagcaacgcgaagaaccttaccaggtcttgacatcctttgaccactctagagatagagctttcccttcggggacaaagtgacaggtggtgcatggttgtcgtcagctcgtgtcgtgagatgttgggttaagtcccgcaacgagcgcaacccttattgttagttgccatcatttagttgggcactctagcgagactgccggtgacaaaccggaggaaggtggggatgacgtcaaatcatcatgccccttatgacctgggctacacacgtgctacaatgggaagtacaacgagtcgctagaccgcgaggtcatgcaaatctcttaaagcttctctcagttcggattgcaggctgcaactcgcctgcatgaagccggaatcgctagtaatcgcggatcagcacgccgcggtgaatacgttcccgggccttgtacacaccgcc